European Patent Specification EP 3 836 975 B1, published July 9, 2025. Title: Nucleic Acid Decontamination Methods. Applicant: Cepheid Kutyavin, Alex I. Lund, Kevin P. Nanassy, Oliver Z. Gall, Alexander A. Brabant, William. The sequence listing filed with the application follows.

SEQUENCE LISTING (4 sequences)

SEQ ID NO: 1 - DNA, 21 bp, Artificial sequence
  Synthetic
agcctggatgacaatgactct

SEQ ID NO: 2 - DNA, 19 bp, Artificial sequence
  Synthetic
cttatgcatgtccttcttg

SEQ ID NO: 3 - DNA, 27 bp, Artificial sequence
  Synthetic
  misc_feature (12)..(12): N at position 12 is Dabcyl-labeled cytosine
cgacggcaacgncaggaggaactacga

SEQ ID NO: 4 - DNA, 126 bp, Salmo
agcctggatgacaatgactctcagcatctgcccccctacgggaactacttccagaacctggggggcgacggcaacgtcaggaggaactacgaactgttggcctgcttcaagaaggacatgcataag